European Patent Application EP 4 268 830 A1, published November 1, 2023. Title: A PHARMACEUTICAL COMPOSITION. Applicant: RIKEN. The sequence listing filed with the application follows.

SEQUENCE LISTING (23 sequences)

SEQ ID NO: 1 - DNA, 15 bp, Artificial Sequence
  Five (5) CAG repeats
cagcagcagcagcag

SEQ ID NO: 2 - DNA, 18 bp, Artificial Sequence
  Six (6) CAG repeats
cagcagcagcagcagcag

SEQ ID NO: 3 - DNA, 21 bp, Artificial Sequence
  Seven (7) CAG repeats
cagcagcagcagcagcagcag

SEQ ID NO: 4 - DNA, 24 bp, Artificial Sequence
  Eight (8) CAG repeats
cagcagcagcagcagcagcagcag

SEQ ID NO: 5 - DNA, 27 bp, Artificial Sequence
  Nine (9) CAG repeats
cagcagcagcagcagcagcagcagcag

SEQ ID NO: 6 - DNA, 30 bp, Artificial Sequence
  Ten (10) CAG repeats
cagcagcagcagcagcagcagcagcagcag

SEQ ID NO: 7 - DNA, 33 bp, Artificial Sequence
  Eleven (11) CAG repeats
cagcagcagcagcagcagcagcagcagcagcag

SEQ ID NO: 8 - DNA, 36 bp, Artificial Sequence
  Twelve (12) CAG repeats
cagcagcagcagcagcagcagcagcagcagcagcag

SEQ ID NO: 9 - DNA, 39 bp, Artificial Sequence
  Thirteen (13) CAG repeats
cagcagcagcagcagcagcagcagcagcagcagcagcag

SEQ ID NO: 10 - DNA, 20 bp, Unknown
  Control antisense oligonucleotide for human DMPK expression (ASO-C)
cctataggactatccaggaa

SEQ ID NO: 11 - DNA, 21 bp, Homo sapiens
ggagtcgaagacagttctagg

SEQ ID NO: 12 - DNA, 20 bp, Homo sapiens
cggagcggttgtgaactggc

SEQ ID NO: 13 - DNA, 21 bp, Homo sapiens
ggtacacaggactggagctgg

SEQ ID NO: 14 - DNA, 16 bp, Homo sapiens
acaataaataccgagg

SEQ ID NO: 15 - DNA, 20 bp, Artificial Sequence
  FAM-P1-F, a forward primer for triplet repeat primed PCR
ggggctcgaagggtccttgt

SEQ ID NO: 16 - DNA, 21 bp, Artificial Sequence
  P2-R, a forward primer for triplet repeat primed PCR
gtgcgtggaggatggaacacg

SEQ ID NO: 17 - DNA, 24 bp, Artificial Sequence
  P3, a forward primer for triplet repeat primed PCR
agcggataacaatttcacacagga

SEQ ID NO: 18 - DNA, 42 bp, Artificial Sequence
  P4-(CAG)6-R, a forward primer for triplet repeat primed PCR
agcggataacaatttcacacaggacagcagcagcagcagcag

SEQ ID NO: 19 - DNA, 20 bp, Artificial Sequence
  P1-F, a reverse primer for triplet repeat primed PCR
ggggctcgaagggtccttgt

SEQ ID NO: 20 - DNA, 21 bp, Artificial Sequence
  HX-P2-R, a reverse primer for triplet repeat primed PCR
gtgcgtggaggatggaacacg

SEQ ID NO: 21 - DNA, 24 bp, Artificial Sequence
  P3, a reverse primer for triplet repeat primed PCR
agcggataacaatttcacacagga

SEQ ID NO: 22 - DNA, 44 bp, Artificial Sequence
  P4(CTG)6-F, a reverse primer for triplet repeat primed PCR
agaggataacaatttcacacaggatgctgctgctgctgctgctg

SEQ ID NO: 23 - DNA, 21 bp, Artificial Sequence
  nucleotide sequence for control ASO
cacgcgagacacgcgagacga